European Patent Application EP 4 495 247 A1, published January 22, 2025. Title: Virus particle comprising capside poteins lingked by linker. Applicant: Denka Company Limited. Application JP. The sequence listing filed with the application follows.

SEQUENCE LISTING (12 sequences)

SEQ ID NO: 1 - protein, 5 aa, synthetic construct
  REGION 1..5: note = peptide linker
GGGGS

SEQ ID NO: 2 - DNA, 1620 bp, Norovirus GII
  source 1..1620: mol_type = genomic DNA
atgaagatggcgtcgagtgacgccaacccatctgatgggtccacagccaacctcgtcccagaggtcaacaatgaggttatggctttggagcccgttgttggtgccgctattgcggcacctgtagcgggccaacaaaatgtaattgacccctggattagaaataattttgtacaagcccctggtggagagtttacagtatcccctagaaacgctccaggtgaaatactatggagcgcgcccttgggccctgatttgaatccctacctttcccatttggccagaatgtacaatagttatgcaggtggttttgaagtgcaggtaatccttgcggggaacgcgttcaccgccggaaaaatcatatttgcagcagtcccaccaaatttcccaactgaaggcttgagccccagccaggtcactatgttcccccatataatagtagatgttaggcaactggaacctgtgttgattcctttacccgatgttaggaataatttctatcactacaatcaatcaaacgaccccaccatcaaattgatagcaatgttgtacacaccacttagggctaataatgctggggacgatgtcttcacagtttcttgtcgggttctcacgagaccatcccccgattttgatttcatatttttagtgccacccacagttgagtcaagaactaaaccattctctgtcccaattttaactgttgaggagatgaccaattcaagattccccattcctttggaaaagttgttcacgggtcccagcagtgcctttgttgttcaaccacaaaatggcaggtgcacgactgatggcgtgctcttaggtactacccaactgtctcctgtcaacatctgcaccttcagaggggatgtcacccacattgctggtactcaagaatacacaatgaatctggcctcccaaaactggaacaattatgacccaacagaagaaatcccagcccctctgggaactccagatttcgtgggtaagatccaaggcgtgctcacccaaaccacaaggagggatggctcgacccgcggtcacaaagccacagtgagcactggaagtgtccacttcaccccaaagctgggcagaattcaattctccactgatacaagcaatgattttgaaactggccaaaacacgagattcaccccagtcggtgttgtccaggatggtagtaccacccaccaaaatgaaccccaacaatgggtactcccaaattattcaggtagagatagtcacaatgtgcacctagcccctgccgtggccccctcttttccgggtgagcaacttcttttcttcaggtccactatgcccggatgcagcgggtatcccaacatgaatttggattgtctactcccccaggagtgggtgcagcacttctaccaagaggcagccccagcacaatctgatgtggctctgctaagatttgtgaatccagacacaggtagggttttgtttgagtgtaagcttcataaatcaggctatgtcacagtggctcacactggccaacatgatttagttatcccccccaatggctattttagatttgattcctgggtcaaccagttctacacacttgcccccatgggaaatgggacggggcgtagacgtgcatta

SEQ ID NO: 3 - DNA, 1620 bp, Norovirus GII
  source 1..1620: mol_type = genomic DNA
aagatggcgtcgagtgacgccaacccatctgatgggtccgcagccaacctcgtaccagaggtcaataatgaggttatggctttggagcccgttgttggtgccgctattgcggcacctgtagcgggccaacaaaatgtaattgacccctggattagaaataattttgtacaagcccctggtggagagtttacagtatcccctagaaacgctccaggtgaaatactatggagcgcgcccctaggccctgacctaaacccctatctatcccatttggccagaatgtacaatggttatgcaggtggttttgaagtgcaggtaattctcgcggggaacgcgttcaccgccgggaagatcatatttgcagcagtcccaccaaattttccaactgaaggcttaagccctagccaggtcactatgttcccccatataatagtagatgttagacaattagaacctgtgctgattcccttacccgatgtcaggaataatttctatcattataatcaatcaaatgattccactattaagttgatagcaatgttgtatacaccacttagggctaataatgctggggatgatgttttcacagtttcgtgccgagttctcacgagaccatcccccgattttgattttatatttttagtgccacccacagttgaatcaagaactaaaccattctctgtcccagttttaactgttgaggagatgaccaattcaagattccccattcctttggaaaagttgttcacgggccccagcagtgcctttgttgttcaaccacaaaacggcaggtgcacaactgatggcgtgctcctaggcaccacccaactgtctcctgtcaacatctgcaccttcagaggggatgtcacccacatcacaggtagtcgcaactacacaatgaatttggcttcccaaaattggaataactatgacccaacagaagaaatcccagcccctctgggaactccagattttgtggggaagattcaaggcatgctcactcaaaccacaaggacagatggttcaacacgcggccacaaagctacagtgtacactgggagcgccgactttgctccaaaactgggtagagttcaatttgaaactgacacagaccatgattttgaagctaaccaaaacacaaagttcaccccagtcggtgtcatccaagatggtagcaccacccaccgaaacgaaccccaacagtgggtgctcccaagttactcaggcagaaatactcacaatgtacatctggcccccgctgtagcccccacctttccaggtgagcaacttctcttcttcagatccaccatgcccggatgcagcgggtaccccaacatggatttggactgtctgctcccccaggaatgggtgcagtacttctatcaagaggcagccccagcacaatctgatgtggctctgctaagatttgtgaatccagacacaggtagggttttgtttgagtgcaagcttcataaatcaggctatgttacagtggctcacactggccaacatgatttggttatcccccccaatggttactttaggtttgattcctgggtcaaccaattctacacgcttgcccccatgggaaatggaacggggcgtagacgtgtagtataa

SEQ ID NO: 4 - DNA, 60 bp, synthetic construct
  misc_feature 1..60: note = peptide linker
  source 1..60: mol_type = other DNA
ggtggcggaggttcaggtggaggcggtagtggaggtggcggttctggaggcggaggatct

SEQ ID NO: 5 - DNA, 74 bp, synthetic construct
  misc_feature 1..74: note = peptide linker
  source 1..74: mol_type = other DNA
ggtggcggaggttcaggtggaggcggtagtggaggtggcggttctggaggcggaggatctggtggaggaggtag

SEQ ID NO: 6 - DNA, 90 bp, synthetic construct
  misc_feature 1..90: note = peptide linker
  source 1..90: mol_type = other DNA
ggtggcggaggttcaggtggaggcggtagtggaggtggcggttctggaggcggaggatctggtggaggaggtagtggcggtggtggatca

SEQ ID NO: 7 - DNA, 3300 bp, synthetic construct
  misc_feature 1..3300: note = VP1 dimer
  source 1..3300: mol_type = other DNA
atgaagatggcgtcgagtgacgccaacccatctgatgggtccacagccaacctcgtcccagaggtcaacaatgaggttatggctttggagcccgttgttggtgccgctattgcggcacctgtagcgggccaacaaaatgtaattgacccctggattagaaataattttgtacaagcccctggtggagagtttacagtatcccctagaaacgctccaggtgaaatactatggagcgcgcccttgggccctgatttgaatccctacctttcccatttggccagaatgtacaatagttatgcaggtggttttgaagtgcaggtaatccttgcggggaacgcgttcaccgccggaaaaatcatatttgcagcagtcccaccaaatttcccaactgaaggcttgagccccagccaggtcactatgttcccccatataatagtagatgttaggcaactggaacctgtgttgattcctttacccgatgttaggaataatttctatcactacaatcaatcaaacgaccccaccatcaaattgatagcaatgttgtacacaccacttagggctaataatgctggggacgatgtcttcacagtttcttgtcgggttctcacgagaccatcccccgattttgatttcatatttttagtgccacccacagttgagtcaagaactaaaccattctctgtcccaattttaactgttgaggagatgaccaattcaagattccccattcctttggaaaagttgttcacgggtcccagcagtgcctttgttgttcaaccacaaaatggcaggtgcacgactgatggcgtgctcttaggtactacccaactgtctcctgtcaacatctgcaccttcagaggggatgtcacccacattgctggtactcaagaatacacaatgaatctggcctcccaaaactggaacaattatgacccaacagaagaaatcccagcccctctgggaactccagatttcgtgggtaagatccaaggcgtgctcacccaaaccacaaggagggatggctcgacccgcggtcacaaagccacagtgagcactggaagtgtccacttcaccccaaagctgggcagaattcaattctccactgatacaagcaatgattttgaaactggccaaaacacgagattcaccccagtcggtgttgtccaggatggtagtaccacccaccaaaatgaaccccaacaatgggtactcccaaattattcaggtagagatagtcacaatgtgcacctagcccctgccgtggccccctcttttccgggtgagcaacttcttttcttcaggtccactatgcccggatgcagcgggtatcccaacatgaatttggattgtctactcccccaggagtgggtgcagcacttctaccaagaggcagccccagcacaatctgatgtggctctgctaagatttgtgaatccagacacaggtagggttttgtttgagtgtaagcttcataaatcaggctatgtcacagtggctcacactggccaacatgatttagttatcccccccaatggctattttagatttgattcctgggtcaaccagttctacacacttgcccccatgggaaatgggacggggcgtagacgtgcattaggtggcggaggttcaggtggaggcggtagtggaggtggcggttctggaggcggaggatctaagatggcgtcgagtgacgccaacccatctgatgggtccgcagccaacctcgtaccagaggtcaataatgaggttatggctttggagcccgttgttggtgccgctattgcggcacctgtagcgggccaacaaaatgtaattgacccctggattagaaataattttgtacaagcccctggtggagagtttacagtatcccctagaaacgctccaggtgaaatactatggagcgcgcccctaggccctgacctaaacccctatctatcccatttggccagaatgtacaatggttatgcaggtggttttgaagtgcaggtaattctcgcggggaacgcgttcaccgccgggaagatcatatttgcagcagtcccaccaaattttccaactgaaggcttaagccctagccaggtcactatgttcccccatataatagtagatgttagacaattagaacctgtgctgattcccttacccgatgtcaggaataatttctatcattataatcaatcaaatgattccactattaagttgatagcaatgttgtatacaccacttagggctaataatgctggggatgatgttttcacagtttcgtgccgagttctcacgagaccatcccccgattttgattttatatttttagtgccacccacagttgaatcaagaactaaaccattctctgtcccagttttaactgttgaggagatgaccaattcaagattccccattcctttggaaaagttgttcacgggccccagcagtgcctttgttgttcaaccacaaaacggcaggtgcacaactgatggcgtgctcctaggcaccacccaactgtctcctgtcaacatctgcaccttcagaggggatgtcacccacatcacaggtagtcgcaactacacaatgaatttggcttcccaaaattggaataactatgacccaacagaagaaatcccagcccctctgggaactccagattttgtggggaagattcaaggcatgctcactcaaaccacaaggacagatggttcaacacgcggccacaaagctacagtgtacactgggagcgccgactttgctccaaaactgggtagagttcaatttgaaactgacacagaccatgattttgaagctaaccaaaacacaaagttcaccccagtcggtgtcatccaagatggtagcaccacccaccgaaacgaaccccaacagtgggtgctcccaagttactcaggcagaaatactcacaatgtacatctggcccccgctgtagcccccacctttccaggtgagcaacttctcttcttcagatccaccatgcccggatgcagcgggtaccccaacatggatttggactgtctgctcccccaggaatgggtgcagtacttctatcaagaggcagccccagcacaatctgatgtggctctgctaagatttgtgaatccagacacaggtagggttttgtttgagtgcaagcttcataaatcaggctatgttacagtggctcacactggccaacatgatttggttatcccccccaatggttactttaggtttgattcctgggtcaaccaattctacacgcttgcccccatgggaaatggaacggggcgtagacgtgtagtataa

SEQ ID NO: 8 - DNA, 3300 bp, synthetic construct; identical to SEQ ID NO: 7
  misc_feature 1..3300: note = VP1 dimer
  source 1..3300: mol_type = other DNA

SEQ ID NO: 9 - DNA, 3330 bp, synthetic construct
  misc_feature 1..3330: note = VP1 dimer
  source 1..3330: mol_type = other DNA
atgaagatggcgtcgagtgacgccaacccatctgatgggtccacagccaacctcgtcccagaggtcaacaatgaggttatggctttggagcccgttgttggtgccgctattgcggcacctgtagcgggccaacaaaatgtaattgacccctggattagaaataattttgtacaagcccctggtggagagtttacagtatcccctagaaacgctccaggtgaaatactatggagcgcgcccttgggccctgatttgaatccctacctttcccatttggccagaatgtacaatagttatgcaggtggttttgaagtgcaggtaatccttgcggggaacgcgttcaccgccggaaaaatcatatttgcagcagtcccaccaaatttcccaactgaaggcttgagccccagccaggtcactatgttcccccatataatagtagatgttaggcaactggaacctgtgttgattcctttacccgatgttaggaataatttctatcactacaatcaatcaaacgaccccaccatcaaattgatagcaatgttgtacacaccacttagggctaataatgctggggacgatgtcttcacagtttcttgtcgggttctcacgagaccatcccccgattttgatttcatatttttagtgccacccacagttgagtcaagaactaaaccattctctgtcccaattttaactgttgaggagatgaccaattcaagattccccattcctttggaaaagttgttcacgggtcccagcagtgcctttgttgttcaaccacaaaatggcaggtgcacgactgatggcgtgctcttaggtactacccaactgtctcctgtcaacatctgcaccttcagaggggatgtcacccacattgctggtactcaagaatacacaatgaatctggcctcccaaaactggaacaattatgacccaacagaagaaatcccagcccctctgggaactccagatttcgtgggtaagatccaaggcgtgctcacccaaaccacaaggagggatggctcgacccgcggtcacaaagccacagtgagcactggaagtgtccacttcaccccaaagctgggcagaattcaattctccactgatacaagcaatgattttgaaactggccaaaacacgagattcaccccagtcggtgttgtccaggatggtagtaccacccaccaaaatgaaccccaacaatgggtactcccaaattattcaggtagagatagtcacaatgtgcacctagcccctgccgtggccccctcttttccgggtgagcaacttcttttcttcaggtccactatgcccggatgcagcgggtatcccaacatgaatttggattgtctactcccccaggagtgggtgcagcacttctaccaagaggcagccccagcacaatctgatgtggctctgctaagatttgtgaatccagacacaggtagggttttgtttgagtgtaagcttcataaatcaggctatgtcacagtggctcacactggccaacatgatttagttatcccccccaatggctattttagatttgattcctgggtcaaccagttctacacacttgcccccatgggaaatgggacggggcgtagacgtgcattaggtggcggaggttcaggtggaggcggtagtggaggtggcggttctggaggcggaggatctggtggaggaggtagtggcggtggtggatcaaagatggcgtcgagtgacgccaacccatctgatgggtccgcagccaacctcgtaccagaggtcaataatgaggttatggctttggagcccgttgttggtgccgctattgcggcacctgtagcgggccaacaaaatgtaattgacccctggattagaaataattttgtacaagcccctggtggagagtttacagtatcccctagaaacgctccaggtgaaatactatggagcgcgcccctaggccctgacctaaacccctatctatcccatttggccagaatgtacaatggttatgcaggtggttttgaagtgcaggtaattctcgcggggaacgcgttcaccgccgggaagatcatatttgcagcagtcccaccaaattttccaactgaaggcttaagccctagccaggtcactatgttcccccatataatagtagatgttagacaattagaacctgtgctgattcccttacccgatgtcaggaataatttctatcattataatcaatcaaatgattccactattaagttgatagcaatgttgtatacaccacttagggctaataatgctggggatgatgttttcacagtttcgtgccgagttctcacgagaccatcccccgattttgattttatatttttagtgccacccacagttgaatcaagaactaaaccattctctgtcccagttttaactgttgaggagatgaccaattcaagattccccattcctttggaaaagttgttcacgggccccagcagtgcctttgttgttcaaccacaaaacggcaggtgcacaactgatggcgtgctcctaggcaccacccaactgtctcctgtcaacatctgcaccttcagaggggatgtcacccacatcacaggtagtcgcaactacacaatgaatttggcttcccaaaattggaataactatgacccaacagaagaaatcccagcccctctgggaactccagattttgtggggaagattcaaggcatgctcactcaaaccacaaggacagatggttcaacacgcggccacaaagctacagtgtacactgggagcgccgactttgctccaaaactgggtagagttcaatttgaaactgacacagaccatgattttgaagctaaccaaaacacaaagttcaccccagtcggtgtcatccaagatggtagcaccacccaccgaaacgaaccccaacagtgggtgctcccaagttactcaggcagaaatactcacaatgtacatctggcccccgctgtagcccccacctttccaggtgagcaacttctcttcttcagatccaccatgcccggatgcagcgggtaccccaacatggatttggactgtctgctcccccaggaatgggtgcagtacttctatcaagaggcagccccagcacaatctgatgtggctctgctaagatttgtgaatccagacacaggtagggttttgtttgagtgcaagcttcataaatcaggctatgttacagtggctcacactggccaacatgatttggttatcccccccaatggttactttaggtttgattcctgggtcaaccaattctacacgcttgcccccatgggaaatggaacggggcgtagacgtgtagtataa

SEQ ID NO: 10 - protein, 1139 aa, synthetic construct
  REGION 1..1139: note = VP1 dimer
MKMASSDANPSDGSTANLVPEVNNEVMALEPVVGAAIAAPVAGQQNVIDPWIRNNFVQAPGGEFTVSPRNAPGEILWSAPLGPDLNPYLSHLARMYNSYAGGFEVQVILAGNAFTAGKIIFAAVPPNFPTEGLSPSQVTMFPHIIVDVRQLEPVLIPLPDVRNNFYHYNQSNDPTIKLIAMLYTPLRANNAGDDVFTVSCRVLTRPSPDFDFIFLVPPTVESRTKPFSVPILTVEEMTNSRFPIPLEKLFTGPSSAFVVQPQNGRCTTDGVLLGTTQLSPVNICTFRGDVTHIAGTQEYTMNLASQNWNNYDPTEEIPAPLGTPDFVGKIQGVLTQTTRRDGSTRGHKATVSTGSVHFTPKLGRIQFSTDTSNDFETGQNTRFTPVGVVQDGSTTHQNEPQQWVLPNYSGRDSHNVHLAPAVAPSFPGEQLLFFRSTMPGCSGYPNMNLDCLLPQEWVQHFYQEAAPAQSDVALLRFVNPDTGRVLFECKLHKSGYVTVAHTGQHDLVIPPNGYFRFDSWVNQFYTLAPMGNGTGRRRALGGTGGCGGAGGTTCAGGTGGAGGCGGTAGTGGAGGTGGCGGTTCTGGAGGCGGAGGATCTKMASSDANPSDGSAANLVPEVNNEVMALEPVVGAAIAAPVAGQQNVIDPWIRNNFVQAPGGEFTVSPRNAPGEILWSAPLGPDLNPYLSHLARMYNGYAGGFEVQVILAGNAFTAGKIIFAAVPPNFPTEGLSPSQVTMFPHIIVDVRQLEPVLIPLPDVRNNFYHYNQSNDSTIKLIAMLYTPLRANNAGDDVFTVSCRVLTRPSPDFDFIFLVPPTVESRTKPFSVPVLTVEEMTNSRFPIPLEKLFTGPSSAFVVQPQNGRCTTDGVLLGTTQLSPVNICTFRGDVTHITGSRNYTMNLASQNWNNYDPTEEIPAPLGTPDFVGKIQGMLTQTTRTDGSTRGHKATVYTGSADFAPKLGRVQFETDTDHDFEANQNTKFTPVGVIQDGSTTHRNEPQQWVLPSYSGRNTHNVHLAPAVAPTFPGEQLLFFRSTMPGCSGYPNMDLDCLLPQEWVQYFYQEAAPAQSDVALLRFVNPDTGRVLFECKLHKSGYVTVAHTGQHDLVIPPNGYFRFDSWVNQFYTLAPMGNGTGRRRVV

SEQ ID NO: 11 - protein, 1154 aa, synthetic construct
  REGION 1..1154: note = VP1 dimer
MKMASSDANPSDGSTANLVPEVNNEVMALEPVVGAAIAAPVAGQQNVIDPWIRNNFVQAPGGEFTVSPRNAPGEILWSAPLGPDLNPYLSHLARMYNSYAGGFEVQVILAGNAFTAGKIIFAAVPPNFPTEGLSPSQVTMFPHIIVDVRQLEPVLIPLPDVRNNFYHYNQSNDPTIKLIAMLYTPLRANNAGDDVFTVSCRVLTRPSPDFDFIFLVPPTVESRTKPFSVPILTVEEMTNSRFPIPLEKLFTGPSSAFVVQPQNGRCTTDGVLLGTTQLSPVNICTFRGDVTHIAGTQEYTMNLASQNWNNYDPTEEIPAPLGTPDFVGKIQGVLTQTTRRDGSTRGHKATVSTGSVHFTPKLGRIQFSTDTSNDFETGQNTRFTPVGVVQDGSTTHQNEPQQWVLPNYSGRDSHNVHLAPAVAPSFPGEQLLFFRSTMPGCSGYPNMNLDCLLPQEWVQHFYQEAAPAQSDVALLRFVNPDTGRVLFECKLHKSGYVTVAHTGQHDLVIPPNGYFRFDSWVNQFYTLAPMGNGTGRRRALGGTGGCGGAGGTTCAGGTGGAGGCGGTAGTGGAGGTGGCGGTTCTGGAGGCGGAGGATCTGGTGGAGGAGGTAGTKMASSDANPSDGSAANLVPEVNNEVMALEPVVGAAIAAPVAGQQNVIDPWIRNNFVQAPGGEFTVSPRNAPGEILWSAPLGPDLNPYLSHLARMYNGYAGGFEVQVILAGNAFTAGKIIFAAVPPNFPTEGLSPSQVTMFPHIIVDVRQLEPVLIPLPDVRNNFYHYNQSNDSTIKLIAMLYTPLRANNAGDDVFTVSCRVLTRPSPDFDFIFLVPPTVESRTKPFSVPVLTVEEMTNSRFPIPLEKLFTGPSSAFVVQPQNGRCTTDGVLLGTTQLSPVNICTFRGDVTHITGSRNYTMNLASQNWNNYDPTEEIPAPLGTPDFVGKIQGMLTQTTRTDGSTRGHKATVYTGSADFAPKLGRVQFETDTDHDFEANQNTKFTPVGVIQDGSTTHRNEPQQWVLPSYSGRNTHNVHLAPAVAPTFPGEQLLFFRSTMPGCSGYPNMDLDCLLPQEWVQYFYQEAAPAQSDVALLRFVNPDTGRVLFECKLHKSGYVTVAHTGQHDLVIPPNGYFRFDSWVNQFYTLAPMGNGTGRRRVV

SEQ ID NO: 12 - protein, 1169 aa, synthetic construct
  REGION 1..1169: note = VP1 dimer
MKMASSDANPSDGSTANLVPEVNNEVMALEPVVGAAIAAPVAGQQNVIDPWIRNNFVQAPGGEFTVSPRNAPGEILWSAPLGPDLNPYLSHLARMYNSYAGGFEVQVILAGNAFTAGKIIFAAVPPNFPTEGLSPSQVTMFPHIIVDVRQLEPVLIPLPDVRNNFYHYNQSNDPTIKLIAMLYTPLRANNAGDDVFTVSCRVLTRPSPDFDFIFLVPPTVESRTKPFSVPILTVEEMTNSRFPIPLEKLFTGPSSAFVVQPQNGRCTTDGVLLGTTQLSPVNICTFRGDVTHIAGTQEYTMNLASQNWNNYDPTEEIPAPLGTPDFVGKIQGVLTQTTRRDGSTRGHKATVSTGSVHFTPKLGRIQFSTDTSNDFETGQNTRFTPVGVVQDGSTTHQNEPQQWVLPNYSGRDSHNVHLAPAVAPSFPGEQLLFFRSTMPGCSGYPNMNLDCLLPQEWVQHFYQEAAPAQSDVALLRFVNPDTGRVLFECKLHKSGYVTVAHTGQHDLVIPPNGYFRFDSWVNQFYTLAPMGNGTGRRRALGGTGGCGGAGGTTCAGGTGGAGGCGGTAGTGGAGGTGGCGGTTCTGGAGGCGGAGGATCTGGTGGAGGAGGTAGTGGCGGTGGTGGATCAKMASSDANPSDGSAANLVPEVNNEVMALEPVVGAAIAAPVAGQQNVIDPWIRNNFVQAPGGEFTVSPRNAPGEILWSAPLGPDLNPYLSHLARMYNGYAGGFEVQVILAGNAFTAGKIIFAAVPPNFPTEGLSPSQVTMFPHIIVDVRQLEPVLIPLPDVRNNFYHYNQSNDSTIKLIAMLYTPLRANNAGDDVFTVSCRVLTRPSPDFDFIFLVPPTVESRTKPFSVPVLTVEEMTNSRFPIPLEKLFTGPSSAFVVQPQNGRCTTDGVLLGTTQLSPVNICTFRGDVTHITGSRNYTMNLASQNWNNYDPTEEIPAPLGTPDFVGKIQGMLTQTTRTDGSTRGHKATVYTGSADFAPKLGRVQFETDTDHDFEANQNTKFTPVGVIQDGSTTHRNEPQQWVLPSYSGRNTHNVHLAPAVAPTFPGEQLLFFRSTMPGCSGYPNMDLDCLLPQEWVQYFYQEAAPAQSDVALLRFVNPDTGRVLFECKLHKSGYVTVAHTGQHDLVIPPNGYFRFDSWVNQFYTLAPMGNGTGRRRVV